European Patent Application EP 4 678 727 A2, published January 14, 2026. Title: HEPATO-BILIARY-PANCREATIC TISSUES AND METHODS OF MAKING SAME. Applicant: CHILDREN'S HOSPITAL MEDICAL CENTER, et al. Application EP. The sequence listing filed with the application follows.

SEQUENCE LISTING (52 sequences)

SEQ ID NO: 1 - DNA, 21 bp, synthetic construct
  misc_feature 1..21: note = SOX2 5'Primer
  source 1..21: mol_type = other DNA
gggggaatggaccttgtatag

SEQ ID NO: 2 - DNA, 20 bp, synthetic construct
  misc_feature 1..20: note = SOX2 3'Primer
  source 1..20: mol_type = other DNA
gcaaagctcctaccgtacca

SEQ ID NO: 3 - DNA, 19 bp, synthetic construct
  misc_feature 1..19: note = CDX2 5'Primer
  source 1..19: mol_type = other DNA
atcaccatccggaggaaag

SEQ ID NO: 4 - DNA, 20 bp, synthetic construct
  misc_feature 1..20: note = CDX2 3'Primer
  source 1..20: mol_type = other DNA
tgcggttctgaaaccagatt

SEQ ID NO: 5 - DNA, 18 bp, synthetic construct
  misc_feature 1..18: note = PDX1 5'Primer
  source 1..18: mol_type = other DNA
aagctcacgcgtggaaag

SEQ ID NO: 6 - DNA, 22 bp, synthetic construct
  misc_feature 1..22: note = PDX1 3'Primer
  source 1..22: mol_type = other DNA
gccgtgagatgtacttgttgaa

SEQ ID NO: 7 - DNA, 19 bp, synthetic construct
  misc_feature 1..19: note = HHEX 5'Primer
  source 1..19: mol_type = other DNA
cggacggtgaacgactaca

SEQ ID NO: 8 - DNA, 21 bp, synthetic construct
  misc_feature 1..21: note = HHEX 3'Primer
  source 1..21: mol_type = other DNA
agaaggggctccagagtagag

SEQ ID NO: 9 - DNA, 20 bp, synthetic construct
  misc_feature 1..20: note = ALDH1A2 5'Primer
  source 1..20: mol_type = other DNA
ccacagtgttttccaacgtc

SEQ ID NO: 10 - DNA, 18 bp, synthetic construct
  misc_feature 1..18: note = ALDH1A2 3'Primer
  source 1..18: mol_type = other DNA
tcctgaacagggccaaag

SEQ ID NO: 11 - DNA, 18 bp, synthetic construct
  misc_feature 1..18: note = CYP26A1 5'Primer
  source 1..18: mol_type = other DNA
cgagcactcgtgggagag

SEQ ID NO: 12 - DNA, 20 bp, synthetic construct
  misc_feature 1..20: note = CYP26A1 3'Primer
  source 1..20: mol_type = other DNA
ccaaagaggagttcggttga

SEQ ID NO: 13 - DNA, 18 bp, synthetic construct
  misc_feature 1..18: note = RARA 5'Primer
  source 1..18: mol_type = other DNA
gccatctgcctcatctgc

SEQ ID NO: 14 - DNA, 20 bp, synthetic construct
  misc_feature 1..20: note = RARA 3'Primer
  source 1..20: mol_type = other DNA
tccgcacgtagacctttagc

SEQ ID NO: 15 - DNA, 18 bp, synthetic construct
  misc_feature 1..18: note = RARB 5'Primer
  source 1..18: mol_type = other DNA
ccgaaaagctcaccagga

SEQ ID NO: 16 - DNA, 19 bp, synthetic construct
  misc_feature 1..19: note = RARB 3'Primer
  source 1..19: mol_type = other DNA
cgatggtcagcactggaat

SEQ ID NO: 17 - DNA, 20 bp, synthetic construct
  misc_feature 1..20: note = RARG 5'Primer
  source 1..20: mol_type = other DNA
cagccctacatgttcccaag

SEQ ID NO: 18 - DNA, 20 bp, synthetic construct
  misc_feature 1..20: note = RARG 3'Primer
  source 1..20: mol_type = other DNA
ggcctggaatctccatcttc

SEQ ID NO: 19 - DNA, 22 bp, synthetic construct
  misc_feature 1..22: note = HES1 5'Primer
  source 1..22: mol_type = other DNA
tgccagctgatataatggagaa

SEQ ID NO: 20 - DNA, 25 bp, synthetic construct
  misc_feature 1..25: note = HES1 3'Primer
  source 1..25: mol_type = other DNA
ctccataataggctttgatgacttt

SEQ ID NO: 21 - DNA, 22 bp, synthetic construct
  misc_feature 1..22: note = INS 5'Primer
  source 1..22: mol_type = other DNA
aggcttcttctacacacccaag

SEQ ID NO: 22 - DNA, 18 bp, synthetic construct
  misc_feature 1..18: note = INS 3'Primer
  source 1..18: mol_type = other DNA
cacaatgccacgcttctg

SEQ ID NO: 23 - DNA, 19 bp, synthetic construct
  misc_feature 1..19: note = GCG 5'Primer
  source 1..19: mol_type = other DNA
gtacaaggcagctggcaac

SEQ ID NO: 24 - DNA, 21 bp, synthetic construct
  misc_feature 1..21: note = GCG 3'Primer
  source 1..21: mol_type = other DNA
tgggaagctgagaatgatctg

SEQ ID NO: 25 - DNA, 19 bp, synthetic construct
  misc_feature 1..19: note = NKX2-2 5'Primer
  source 1..19: mol_type = other DNA
cgagggccttcagtactcc

SEQ ID NO: 26 - DNA, 19 bp, synthetic construct
  misc_feature 1..19: note = NKX2-2 3'Primer
  source 1..19: mol_type = other DNA
ggggacttggagcttgagt

SEQ ID NO: 27 - DNA, 22 bp, synthetic construct
  misc_feature 1..22: note = CPA1 5'Primer
  source 1..22: mol_type = other DNA
cagcatcatcaaggcaatttat

SEQ ID NO: 28 - DNA, 19 bp, synthetic construct
  misc_feature 1..19: note = CPA1 3'Primer
  source 1..19: mol_type = other DNA
ggagctcgaaggtgaagga

SEQ ID NO: 29 - DNA, 19 bp, synthetic construct
  misc_feature 1..19: note = CEL 5'Primer
  source 1..19: mol_type = other DNA
ggagctcgaaggtgaagga

SEQ ID NO: 30 - DNA, 21 bp, synthetic construct
  misc_feature 1..21: note = CEL 3'Primer
  source 1..21: mol_type = other DNA
gatcccgaaggccatagttac

SEQ ID NO: 31 - DNA, 26 bp, synthetic construct
  misc_feature 1..26: note = CFTR 5'Primer
  source 1..26: mol_type = other DNA
gaagtagtgatggagaatgtaacagc

SEQ ID NO: 32 - DNA, 23 bp, synthetic construct
  misc_feature 1..23: note = CFTR 3'Primer
  source 1..23: mol_type = other DNA
gctttctcaaataattccccaaa

SEQ ID NO: 33 - DNA, 21 bp, synthetic construct
  misc_feature 1..21: note = CAPN6 5'Primer
  source 1..21: mol_type = other DNA
aggctgctataacaaccgtga

SEQ ID NO: 34 - DNA, 20 bp, synthetic construct
  misc_feature 1..20: note = CAPN6 3'Primer
  source 1..20: mol_type = other DNA
catcctcaggcacagtgaag

SEQ ID NO: 35 - DNA, 20 bp, synthetic construct
  misc_feature 1..20: note = ALB 5'Primer
  source 1..20: mol_type = other DNA
gtgaggttgctcatcggttt

SEQ ID NO: 36 - DNA, 20 bp, synthetic construct
  misc_feature 1..20: note = ALB 3'Primer
  source 1..20: mol_type = other DNA
gagcaaaggcaatcaacacc

SEQ ID NO: 37 - DNA, 18 bp, synthetic construct
  misc_feature 1..18: note = CYP3A7 5'Primer
  source 1..18: mol_type = other DNA
caaacttggccgtggaaa

SEQ ID NO: 38 - DNA, 20 bp, synthetic construct
  misc_feature 1..20: note = CYP3A7 3'Primer
  source 1..20: mol_type = other DNA
agtccatgtgtacgggttcc

SEQ ID NO: 39 - DNA, 21 bp, synthetic construct
  misc_feature 1..21: note = HNF4A 5'Primer
  source 1..21: mol_type = other DNA
gagatccatggtgttcaagga

SEQ ID NO: 40 - DNA, 20 bp, synthetic construct
  misc_feature 1..20: note = HNF4A 3'Primer
  source 1..20: mol_type = other DNA
gtgccgagggacaatgtagt

SEQ ID NO: 41 - DNA, 27 bp, synthetic construct
  misc_feature 1..27: note = AFP 5'Primer
  source 1..27: mol_type = other DNA
tgtactgcagagataagtttagctgac

SEQ ID NO: 42 - DNA, 23 bp, synthetic construct
  misc_feature 1..23: note = AFP 3'Primer
  source 1..23: mol_type = other DNA
tccttgtaagtggcttcttgaac

SEQ ID NO: 43 - DNA, 20 bp, synthetic construct
  misc_feature 1..20: note = APOA2 5'Primer
  source 1..20: mol_type = other DNA
gagaaggtcaagagcccaga

SEQ ID NO: 44 - DNA, 20 bp, synthetic construct
  misc_feature 1..20: note = APOA2 3'Primer
  source 1..20: mol_type = other DNA
ccttcttgatcaggggtgtc

SEQ ID NO: 45 - DNA, 43 bp, Homo sapiens
  source 1..43: mol_type = unassigned DNA
gctaccccagccagtgtcaacacgacaccggataaaccaaaga

SEQ ID NO: 46 - DNA, 25 bp, synthetic construct
  misc_feature 1..25: note = hHES1 gRNA1 F
  source 1..25: mol_type = other DNA
caccgatccggtgtcgtgttgacac

SEQ ID NO: 47 - DNA, 25 bp, synthetic construct
  misc_feature 1..25: note = hHES1 gRNA1 R
  source 1..25: mol_type = other DNA
ctaggccacagcacaactgtgcaaa

SEQ ID NO: 48 - DNA, 22 bp, synthetic construct
  misc_feature 1..22: note = hHES1 Seq F
  source 1..22: mol_type = other DNA
accctcagcacttgctcagtag

SEQ ID NO: 49 - DNA, 25 bp, synthetic construct
  misc_feature 1..25: note = hHES1 Seq R
  source 1..25: mol_type = other DNA
tcttcgtcttttctccataataggc

SEQ ID NO: 50 - DNA, 50 bp, synthetic construct
  misc_feature 1..50: note = Modified gene sequence of WT and HES1KO (Del #11)-A
  source 1..50: mol_type = other DNA
aaaaaaaaaaggaaaatgccagctgatataatggagaaaaattcctcgtc

SEQ ID NO: 51 - DNA, 41 bp, synthetic construct
  misc_feature 1..41: note = Modified gene sequence of WT and HES1KO (Del #11)-B
  source 1..41: mol_type = other DNA
cccggtgctaccccagccagtgtcaacacgacaccggataa

SEQ ID NO: 52 - DNA, 15 bp, synthetic construct
  misc_feature 1..15: note = Modified gene sequence of WT and HES1KO (Del #11)-C
  source 1..15: mol_type = other DNA
cacgacaccggataa